European Patent Specification EP 4 126 949 B1, published September 16, 2026. Title: TIE2-BINDING AGENTS AND METHODS OF USE. Applicant: Genentech, Inc. The sequence listing filed with the application follows.

SEQUENCE LISTING (92 sequences)

SEQ ID NO: 1 - protein, 689 aa, Homo sapiens
MFTMTRAMEEALFQHFMHQKLGIAYAIHKPFPFFEGLLDNSIITKRMYMESLEACRNLIPVSRVVHNILTQLERTFNLSLLVTLFSQINLREYPNLVTIYRSFKRVGASYEWQSRDTPILLEAPTGLAEGSSLHTPLALPPPQPPQPSCSPCAPRVSEPGTSSQQSDEILSESPSPSDPVLPLPALIQEGRSTSVTNDKLTSKMNAEEDSEEMPSLLTSTVQVASDNLIPQIRDKEDPQEMPHSPLGSMPEIRDNSPEPNDPEEPQEVSSTPSDKKGKKRKRCIWSTPKRRHKKKSLPGGTASSRHGIQKKLKRVDQVPQKKDDSTCNSTVETRAQKARTECARKSRSEEIIDGTSEMNEGKRSQKTPSTPRRVTQGAASPGHGIQEKLQVVDKVTQRKDDSTWNSEVMMRVQKARTKCARKSRLKEKKKEKDICSSSKRRFQKNIHRRGKPKSDTVDFHCSKLPVTCGEAKGILYKKKMKHGSSVKCIRNEDGTWLTPNEFEVEGKGRNAKNWKRNIRCEGMTLGELLKRKNSDECEVCCQGGQLLCCGTCPRVFHEDCHIPPVEAKRMLWSCTFCRMKRSSGSQQCHHVSKTLERQMQPQDQLIRDYGEPFQEAMWLDLVKERLITEMYTVAWFVRDMRLMFRNHKTFYKASDFGQVGLDLEAEFEKDLKDVLGFHEANDGGFWTLP

SEQ ID NO: 2 - protein, 1124 aa, Macaca fascicularis
MDSLASLVLCGVSLLLSGTVEGAMDLILINSLPLVSDAETSLTCIASGWHPHEPITIGRDFEALMNQHQDPLEVTQDVTREWAKKVVWKREKASKINGAYFCEGRVRGEAIRIRTMKMRQQASFLPATLTMTVDKGDNVNISFKKVLIKEEDAVIYKNGSFIHSVPRHEVPDILEVHLPHAQPQDAGVYSARYIGGNLFTSAFTRLIVRRCEAQKWGPECNRLCTVCVNNGVCHEDTGECICPPGFMGRTCEKACERHTFGRTCKERCSGQDGCKSYVFCLPDPYGCSCATGWKGLQCNEACHHGFYGPDCKLRCSCSNGETCDRFQGCLCSPGRQGLQCEREGIPRMTPKIVDLPDHIEVNSGKFNPICKASGWPLPTNEEMTLVKPDGTVLHPKDFNHTDHFSVAIFTIHRILPPDSGVWVCSANTVAGMVEKPFNISVKVLPKPLNAPNVIDTGHNFAVINISSEPYFGDGPIKSKKLLYKPVNHYEAWRHIQVTNEIVTLNHLEPRTEYELCVQLVRRGEGGEGHPGPVRRFTTASIGLPPPRGLNLLPKSQTTLNLTWQPIFPSSEDDFYVEVERRSVQKSDQQNIKVPGNLTSVLLNNLHPREQYVVRARVNTKAQGEWSEDLTAWTLSDILPPQPENIKISNITHSSAVISWTILDGYSISSITIRYKVQGKNEDQHIDVKIKNATITQYQLKGLEPETAYQVDIFAENNIGSSNPAFSHELVTLPESEAPADLGGGKMLLIAILGSAGMTCLTVLLAFLIILQLKRANVQRRMAQAFQNVREEPAVQFNSGTLALNRKVKNNPDPTIYPVLDWNDIKFQDVIGEGNFGQVLKARIKKDGLRMDAAIKRMKEYASKDDHRDFAGELEVLCKLGHHPNIINLLGACEHRGYLYLAIEYAPHGNLLDFLRKSRVLETDPAFAIANSTASTLSSQQLLHFAADVARGMDYLSQKQFIHRDLAARNILVGENYVAKIADFGLSRGQEVYVKKTMGRLPVRWMAIESLNYSVYTTNSDVWSYGVLLWEIVSLGGTPYCGMTCAELYEKLPQGYRLEKPLNCDDEVFDLMRQCWREKPYERPSFAQILVSLNRMLEERKTYVNTTLYEKFTYAGIDCSAEEAA

SEQ ID NO: 3 - protein, 5 aa, Artificial Sequence
  Synthetic Construct
NTDIS

SEQ ID NO: 4 - protein, 17 aa, Artificial Sequence
  Synthetic Construct
RISPSDGNTYYADSVKG

SEQ ID NO: 5 - protein, 11 aa, Artificial Sequence
  Synthetic Construct
  misc_feature (7)..(7): Xaa is Met, Leu, Lys, Phe, Tyr, Arg, Asn, Gln, His, of Trp
  misc_feature (9)..(9): Xaa is Phe, Tyr, Leu, Gln, Ile, Lys, or His
RTRWASXAXDY

SEQ ID NO: 6 - protein, 11 aa, Artificial Sequence
  Synthetic Construct
RTRWASWAMDY

SEQ ID NO: 7 - protein, 11 aa, Artificial Sequence
  Synthetic Construct
RTRWASWAFDY

SEQ ID NO: 8 - protein, 11 aa, Artificial Sequence
  Synthetic Construct
RASQDVSTAVA

SEQ ID NO: 9 - protein, 7 aa, Artificial Sequence
  Synthetic Construct
SASFLYS

SEQ ID NO: 10 - protein, 9 aa, Artificial Sequence
  Synthetic Construct
QQSYTTPPT

SEQ ID NO: 11 - protein, 30 aa, Artificial Sequence
  Synthetic Construct
EVQLVESGGGLVQPGGSLRLSCAASGFTFS

SEQ ID NO: 12 - protein, 14 aa, Artificial Sequence
  Synthetic Construct
WVRQAPGKGLEWVG

SEQ ID NO: 13 - protein, 32 aa, Artificial Sequence
  Synthetic Construct
RFTISADTSKNTAYLQMNSLRAEDTAVYYCAR

SEQ ID NO: 14 - protein, 9 aa, Artificial Sequence
  Synthetic Construct
QGTLVTVSS

SEQ ID NO: 15 - protein, 23 aa, Artificial Sequence
  Synthetic Construct
DIQMTQSPSSLSASVGDRVTITC

SEQ ID NO: 16 - protein, 15 aa, Artificial Sequence
  Synthetic Construct
WYQQKPGKAPKLLIY

SEQ ID NO: 17 - protein, 32 aa, Artificial Sequence
  Synthetic Construct
GVPSRFSGSGSGTDFTLTISSLQPEDFATYYC

SEQ ID NO: 18 - protein, 9 aa, Artificial Sequence
  Synthetic Construct
FGQGTKVEI

SEQ ID NO: 19 - protein, 120 aa, Artificial Sequence
  Synthetic Construct
  misc_feature (105)..(105): Xaa can be any naturally occurring amino acid
  misc_feature (107)..(107): Xaa can be any naturally occurring amino acid
EVQLVESGGGLVQPGGSLRLSCAASGFTFSNTDISWVRQAPGKGLEWVGRISPSDGNTYYADSVKGRFTISADTSKNTAYLQMNSLRAEDTAVYYCARRTRWASXAXDYWGQGTLVTVSS

SEQ ID NO: 20 - protein, 120 aa, Artificial Sequence
  Synthetic Construct
EVQLVESGGGLVQPGGSLRLSCAASGFTFSNTDISWVRQAPGKGLEWVGRISPSDGNTYYADSVKGRFTISADTSKNTAYLQMNSLRAEDTAVYYCARRTRWASWAFDYWGQGTLVTVSS

SEQ ID NO: 21 - protein, 107 aa, Artificial Sequence
  Synthetic Construct
DIQMTQSPSSLSASVGDRVTITCRASQDVSTAVAWYQQKPGKAPKLLIYSASFLYSGVPSRFSGSGSGTDFTLTISSLQPEDFATYYCQQSYTTPPTFGQGTKVEIK

SEQ ID NO: 22 - protein, 120 aa, Artificial Sequence
  Synthetic Construct
EVQLVESGGGLVQPGGSLRLSCAASGFTFSNTDISWVRQAPGKGLEWVGRISPSDGNTYYADSVKGRFTISADTSKNTAYLQMNSLRAEDTAVYYCARRTRWASWAMDYWGQGTLVTVSS

SEQ ID NO: 23 - protein, 224 aa, Artificial Sequence
  Synthetic Construct
EVQLVESGGGLVQPGGSLRLSCAASGFTFSNTDISWVRQAPGKGLEWVGRISPSDGNTYYADSVKGRFTISADTSKNTAYLQMNSLRAEDTAVYYCARRTRWASWAFDYWGQGTLVTVSSASTKGPSVFPLAPSSKSTSGGTAALGCLVKDYFPEPVTVSWNSGALTSGVHTFPAVLQSSGLYSLSSVVTVPSSSLGTQTYICNVNHKPSNTKVDKKVEPKSCD

SEQ ID NO: 24 - protein, 224 aa, Artificial Sequence
  Synthetic Construct
EVQLVESGGGLVQPGGSLRLSCAASGFTFSNTDISWVRQAPGKGLEWVGRISPSDGNTYYADSVKGRFTISADTSKNTAYLQMNSLRAEDTAVYYCARRTRWASWAMDYWGQGTLVTVSSASTKGPSVFPLAPSSKSTSGGTAALGCLVKDYFPEPVTVSWNSGALTSGVHTFPAVLQSSGLYSLSSVVTVPSSSLGTQTYICNVNHKPSNCKVDKKVEPKSCD

SEQ ID NO: 25 - protein, 214 aa, Artificial Sequence
  Synthetic Construct
DIQMTQSPSSLSASVGDRVTITCRASQDVSTAVAWYQQKPGKAPKLLIYSASFLYSGVPSRFSGSGSGTDFTLTISSLQPEDFATYYCQQSYTTPPTFGQGTKVEIKRTVAAPSVFIFPPSDEQLKSGTASVVCLLNNFYPREAKVQWKVDNALQSGNSQESVTEQDSKDSTYSLSSTLTLSKADYEKHKVYACEVTHQGLSSPVTKSFNRGEC

SEQ ID NO: 26 - protein, 104 aa, Artificial Sequence
  Synthetic Construct
ASTKGPSVFPLAPSSKSTSGGTAALGCLVKDYFPEPVTVSWNSGALTSGVHTFPAVLQSSGLYSLSSVVTVPSSSLGTQTYICNVNHKPSNCKVDKKVEPKSCD

SEQ ID NO: 27 - protein, 107 aa, Artificial Sequence [sequence omitted]

SEQ ID NO: 28 - protein, 5 aa, Artificial Sequence
  Synthetic Construct
SYWIH

SEQ ID NO: 29 - protein, 17 aa, Artificial Sequence
  Synthetic Construct
AISPNDGSTYYADSVKG

SEQ ID NO: 30 - protein, 15 aa, Artificial Sequence
  Synthetic Construct
SRYYGQRLVYYVMDY

SEQ ID NO: 31 - protein, 124 aa, Artificial Sequence
  Synthetic Construct
EVQLVESGGGLVQPGGSLRLSCAASGFTFSSYWIHWVRQAPGKGLEWVAAISPNDGSTYYADSVKGRFTISADTSKNTAYLQMNSLRAEDTAVYYCARSRYYGQRLVYYVMDYWGQGTLVTVSS

SEQ ID NO: 32 - protein, 228 aa, Artificial Sequence
  Synthetic Construct
EVQLVESGGGLVQPGGSLRLSCAASGFTFSSYWIHWVRQAPGKGLEWVAAISPNDGSTYYADSVKGRFTISADTSKNTAYLQMNSLRAEDTAVYYCARSRYYGQRLVYYVMDYWGQGTLVTVSSASTKGPSVFPLAPSSKSTSGGTAALGCLVKDYFPEPVTVSWNSGALTSGVHTFPAVLQSSGLYSLSSVVTVPSSSLGTQTYICNVNHKPSNTKVDKKVEPKSCD

SEQ ID NO: 33 - protein, 5 aa, Artificial Sequence
  Synthetic Construct
SSGIS

SEQ ID NO: 34 - protein, 17 aa, Artificial Sequence
  Synthetic Construct
TINPYGGDTYYADSVKG

SEQ ID NO: 35 - protein, 11 aa, Artificial Sequence
  Synthetic Construct
FYRFLSSGMDY

SEQ ID NO: 36 - protein, 120 aa, Artificial Sequence
  Synthetic Construct
EVQLVESGGGLVQPGGSLRLSCAASGFTFTSSGISWVRQAPGKGLEWVATINPYGGDTYYADSVKGRFTISADTSKNTAYLQMNSLRAEDTAVYYCARFYRFLSSGMDYWGQGTLVTVSS

SEQ ID NO: 37 - protein, 224 aa, Artificial Sequence
  Synthetic Construct
EVQLVESGGGLVQPGGSLRLSCAASGFTFTSSGISWVRQAPGKGLEWVATINPYGGDTYYADSVKGRFTISADTSKNTAYLQMNSLRAEDTAVYYCARFYRFLSSGMDYWGQGTLVTVSSASTKGPSVFPLAPSSKSTSGGTAALGCLVKDYFPEPVTVSWNSGALTSGVHTFPAVLQSSGLYSLSSVVTVPSSSLGTQTYICNVNHKPSNTKVDKKVEPKSCD

SEQ ID NO: 38 - protein, 5 aa, Artificial Sequence
  Synthetic Construct
GSWIS

SEQ ID NO: 39 - protein, 17 aa, Artificial Sequence
  Synthetic Construct
RINPYDGNTYYADSVKG

SEQ ID NO: 40 - protein, 10 aa, Artificial Sequence
  Synthetic Construct
NNRFPTWFDY

SEQ ID NO: 41 - protein, 119 aa, Artificial Sequence
  Synthetic Construct
EVQLVESGGGLVQPGGSLRLSCAASGFTFSGSWISWVRQAPGKGLEWVARINPYDGNTYYADSVKGRFTISADTSKNTAYLQMNSLRAEDTAVYYCARNNRFPTWFDYWGQGTLVTVSS

SEQ ID NO: 42 - protein, 223 aa, Artificial Sequence
  Synthetic Construct
EVQLVESGGGLVQPGGSLRLSCAASGFTFSGSWISWVRQAPGKGLEWVARINPYDGNTYYADSVKGRFTISADTSKNTAYLQMNSLRAEDTAVYYCARNNRFPTWFDYWGQGTLVTVSSASTKGPSVFPLAPSSKSTSGGTAALGCLVKDYFPEPVTVSWNSGALTSGVHTFPAVLQSSGLYSLSSVVTVPSSSLGTQTYICNVNHKPSNTKVDKKVEPKSCD

SEQ ID NO: 43 - protein, 5 aa, Artificial Sequence
  Synthetic Construct
DTYIH

SEQ ID NO: 44 - protein, 17 aa, Artificial Sequence
  Synthetic Construct
VIYPDNGATYYADSVKG

SEQ ID NO: 45 - protein, 10 aa, Artificial Sequence
  Synthetic Construct
EFACARCVYG

SEQ ID NO: 46 - protein, 235 aa, Artificial Sequence
EVQLVESGGGLVQPGGSLRLSCAASGFTFSDTYIHWVRQAPGKGLEWVAVIYPDNGATYYADSVKGTYYADSVKGRFTISADTSKNTAYLQMNSLRAEDTAVYYCAREFACARCVYGMDYWGQGTLVTVSSASTKGPSVFPLAPSSKSTSGGTAALGCLVKDYFPEPVTVSWNSGALTSGVHTFPAVLQSSGLYSLSSVVTVPSSSLGTQTYICNVNHKPSNTKVDKKVEPKSCD

SEQ ID NO: 47 - protein, 131 aa, Artificial Sequence
  Synthetic Construct
EVQLVESGGGLVQPGGSLRLSCAASGFTFSDTYIHWVRQAPGKGLEWVAVIYPDNGATYYADSVKGTYYADSVKGRFTISADTSKNTAYLQMNSLRAEDTAVYYCAREFACARCVYGMDYWGQGTLVTVSS

SEQ ID NO: 48 - protein, 5 aa, Artificial Sequence
  Synthetic Construct
NSAIH

SEQ ID NO: 49 - protein, 17 aa, Artificial Sequence
  Synthetic Construct
SITPYNGYTYYADSVKG

SEQ ID NO: 50 - protein, 10 aa, Artificial Sequence
  Synthetic Construct
RQSYSYVMDY

SEQ ID NO: 51 - protein, 119 aa, Artificial Sequence
  Synthetic Construct
EVQLVESGGGLVQPGGSLRLSCAASGFTFSNSAIHWVRQAPGKGLEWVASITPYNGYTYYADSVKGRFTISADTSKNTAYLQMNSLRAEDTAVYYCARRQSYSYVMDYWGQGTLVTVSS

SEQ ID NO: 52 - protein, 223 aa, Artificial Sequence
  Synthetic Construct
EVQLVESGGGLVQPGGSLRLSCAASGFTFSNSAIHWVRQAPGKGLEWVASITPYNGYTYYADSVKGRFTISADTSKNTAYLQMNSLRAEDTAVYYCARRQSYSYVMDYWGQGTLVTVSSASTKGPSVFPLAPSSKSTSGGTAALGCLVKDYFPEPVTVSWNSGALTSGVHTFPAVLQSSGLYSLSSVVTVPSSSLGTQTYICNVNHKPSNTKVDKKVEPKSCD

SEQ ID NO: 53 - protein, 214 aa, Artificial Sequence; identical to SEQ ID NO: 25
  Synthetic Construct

SEQ ID NO: 54 - protein, 684 aa, Artificial Sequence
  Synthetic Construct
EVQLVESGGGLVQPGGSLRLSCAASGFTFSNTDISWVRQAPGKGLEWVGRISPSDGNTYYADSVKGRFTISADTSKNTAYLQMNSLRAEDTAVYYCARRTRWASWAMDYWGQGTLVTVSSASTKGPSVFPLAPSSKSTSGGTAALGCLVKDYFPEPVTVSWNSGALTSGVHTFPAVLQSSGLYSLSSVVTVPSSSLGTQTYICNVNHKPSNTKVDKKVEPKSCDKTHTGGGGSGGEVQLVESGGGLVQPGGSLRLSCAASGFTFSNSAIHWVRQAPGKGLEWVASITPYNGYTYYADSVKGRFTISADTSKNTAYLQMNSLRAEDTAVYYCARRQSYSYVMDYWGQGTLVTVSSASTKGPSVFPLAPSSKSTSGGTAALGCLVKDYFPEPVTVSWNSGALTSGVHTFPAVLQSSGLYSLSSVVTVPSSSLGTQTYICNVNHKPSNTKVDKKVEPKSCDKTHTCPPCPAPEAAGGPSVFLFPPKPKDTLMASRTPEVTCVVVDVSHEDPEVKFNWYVDGVEVHNAKTKPREEQYNSTYRVVSVLTVLAQDWLNGKEYKCKVSNKALGAPIEKTISKAKGQPREPQVYTLPPSREEMTKNQVSLTCLVKGFYPSDIAVEWESNGQPENNYKTTPPVLDSDGSFFLYSKLTVDKSRWQQGNVFSCSVMHEALHNAYTQKSLSLSPGK

SEQ ID NO: 55 - protein, 224 aa, Artificial Sequence
  Synthetic Construct
EVQLVESGGGLVQPGGSLRLSCAASGFTFSNTDISWVRQAPGKGLEWVGRISPSDGNTYYADSVKGRFTISADTSKNTAYLQMNSLRAEDTAVYYCARRTRWASWAFDYWGQGTLVTVSSASTKGPSVFPLAPSSKSTSGGTAALGCLVKDYFPEPVTVSWNSGALTSGVHTFPAVLQSSGLYSLSSVVTVPSSSLGTQTYICNVNHKPSNCKVDKKVEPKSCD

SEQ ID NO: 56 - protein, 214 aa, Artificial Sequence
  Synthetic Construct
DIQMTQSPSSLSASVGDRVTITCRASQDVSTAVAWYQQKPGKAPKLLIYSASFLYSGVPSRFSGSGSGTDFTLTISSLQPEDFATYYCQQSYTTPPTFGQGTKVEIKRTVAAPSVFIFPPSDEQLKSGTASVVCLLNNFYPREAKVQWKVDNALQSGNSQESVTEQDSKDSTYSLSSTLTLSKADYEKHKVYACEVTHQGLSSPVCKSFNRGEC

SEQ ID NO: 57 - protein, 232 aa, Artificial Sequence
  Synthetic Construct
EVQLVESGGGLVQPGGSLRLSCAASGFTFSNTDISWVRQAPGKGLEWVGRISPSDGNTYYADSVKGRFTISADTSKNTAYLQMNSLRAEDTAVYYCARRTRWASWAFDYWGQGTLVTVSSASTKGPSVFPLAPSSKSTSGGTAALGCLVKDYFPEPVTVSWNSGALTSGVHTFPAVLQSSGLYSLSSVVTVPSSSLGTQTYICNVNHKPSNTKVDKKVEPKSCDKTHTSPPC

SEQ ID NO: 58 - protein, 224 aa, Artificial Sequence
  Synthetic Construct
EVQLVESGGGLVQPGGSLRLSCAASGFTFSNTDISWVRQAPGKGLEWVGRISPSDGNTYYADSVKGRFTISADTSKNTAYLQMNSLRAEDTAVYYCARRTRWASWAFDYWGQGTLVTVSSASCKGPSVFPLAPSSKSTSGGTAALGCLVKDYFPEPVTVSWNSGALTSGVHTFPAVLQSSGLYSLSSVVTVPSSSLGTQTYICNVNHKPSNTKVDKKVEPKSCD

SEQ ID NO: 59 - protein, 224 aa, Artificial Sequence
  Synthetic Construct
EVQLVESGGGLVQPGGSLRLSCAASGFTFSNTDISWVRQAPGKGLEWVGRISPSDGNTYYADSVKGRFTISADTSKNTAYLQMNSLRAEDTAVYYCARRTRWASWAFDYWGQGTLVTVSSASTKGPSVFPLAPSSKSTSGGTAALGCLVKDYFPEPVTVSWNSGALTSCVHTFPAVLQSSGLYSLSSVVTVPSSSLGTQTYICNVNHKPSNTKVDKKVEPKSCD

SEQ ID NO: 60 - protein, 224 aa, Artificial Sequence
  Synthetic Construct
EVQLVESGGGLVQPGGSLRLSCAASGFTFSNTDISWVRQAPGKGLEWVGRISPSDGNTYYADSVKGRFTISADTSKNTAYLQMNSLRAEDTAVYYCARRTRWASWAFDYWGQGTLVTVSSASTKGPSVFPLAPSSKSTSGGTAALGCLVKDYFPEPVTVSWNSGALTSGVHTFPAVLQSSCLYSLSSVVTVPSSSLGTQTYICNVNHKPSNTKVDKKVEPKSCD

SEQ ID NO: 61 - protein, 224 aa, Artificial Sequence
  Synthetic Construct
EVQLVESGGGLVQPGGSLRLSCAASGFTFSNTDISWVRQAPGKGLEWVGRISPSDGNTYYADSVKGRFTISADTSKNTAYLQMNSLRAEDTAVYYCARRTRWASWAFDYWGQGTLVTVSSASTKGPSVFPLAPSSKSTSGGTAALGCLVKDYFPEPVTVSWNSGALTSGVHTFPAVLQSSGLYSLSSVVCVPSSSLGTQTYICNVNHKPSNTKVDKKVEPKSCD

SEQ ID NO: 62 - protein, 214 aa, Artificial Sequence
  Synthetic Construct
DIQMTQSPSSLSASVGDRVTITCRASQDVSTAVAWYQQKPGKAPKLLIYSASFLYSGVPSRFSGSGSGTDFTLTISSLQPEDFATYYCQQSYTTPPTFGQGTKVEIKRTVAAPSVFIFPPSDECLKSGTASVVCLLNNFYPREAKVQWKVDNALQSGNSQESVTEQDSKDSTYSLSSTLTLSKADYEKHKVYACEVTHQGLSSPVTKSFNRGEC

SEQ ID NO: 63 - protein, 214 aa, Artificial Sequence
  Synthetic Construct
DIQMTQSPSSLSASVGDRVTITCRASQDVSTAVAWYQQKPGKAPKLLIYSASFLYSGVPSRFSGSGSGTDFTLTISSLQPEDFATYYCQQSYTTPPTFGQGTKVEIKRTVAAPSVFIFPPSDEQLKSGTASVVCLLNNFYPCEAKVQWKVDNALQSGNSQESVTEQDSKDSTYSLSSTLTLSKADYEKHKVYACEVTHQGLSSPVTKSFNRGEC

SEQ ID NO: 64 - protein, 214 aa, Artificial Sequence
  Synthetic Construct
DIQMTQSPSSLSASVGDRVTITCRASQDVSTAVAWYQQKPGKAPKLLIYSASFLYSGVPSRFSGSGSGTDFTLTISSLQPEDFATYYCQQSYTTPPTFGQGTKVEIKRTVAAPSVFIFPPSDEQLKSGTASVVCLLNNFYPREAKVQWKVDNALCSGNSQESVTEQDSKDSTYSLSSTLTLSKADYEKHKVYACEVTHQGLSSPVTKSFNRGEC

SEQ ID NO: 65 - protein, 214 aa, Artificial Sequence
  Synthetic Construct
DIQMTQSPSSLSASVGDRVTITCRASQDVSTAVAWYQQKPGKAPKLLIYSASFLYSGVPSRFSGSGSGTDFTLTISSLQPEDFATYYCQQSYTTPPTFGQGTKVEIKRTVAAPSVFIFPPSDEQLKSGTASVVCLLNNFYPREAKVQWKVDNALQSGNSQESVTEQDSKDSTYSLSSTLTLSKADYEKHKVYACEVTHQGCSSPVTKSFNRGEC

SEQ ID NO: 66 - protein, 214 aa, Artificial Sequence
  Synthetic Construct
DIQMTQSPSSLSASVGDRVTITCRASQDVSTAVAWYQQKPGKAPKLLIYSASFLYSGVPSRFSGSGSGTDFTLTISSLQPEDFATYYCQQSYTTPPTFGQGTKVEICRTVAAPSVFIFPPSDEQLKSGTASVVCLLNNFYPREAKVQWKVDNALQSGNSQESVTEQDSKDSTYSLSSTLTLSKADYEKHKVYACEVTHQGLSSPVTKSFNRGEC

SEQ ID NO: 67 - protein, 214 aa, Artificial Sequence
  Synthetic Construct
DIQMTQSPSSLSASVGDRVTITCRASQDVSTAVAWYQQKPGKAPKLLIYSASFLYSGVPSRFSGSGSGTDFTLTISSLQPEDFATYYCQQSYTTPPTFGQGTKVEIKRTVAAPSVFIFPPSDEQLCSGTASVVCLLNNFYPREAKVQWKVDNALQSGNSQESVTEQDSKDSTYSLSSTLTLSKADYEKHKVYACEVTHQGLSSPVTKSFNRGEC

SEQ ID NO: 68 - protein, 214 aa, Artificial Sequence
  Synthetic Construct
DIQMTQSPSSLSASVGDRVTITCRASQDVSTAVAWYQQKPGKAPKLLIYSASFLYSGVPSRFSGSGSGTDFTLTISSLQPEDFATYYCQQSYTTPPTFGQGTKVEIKRTVAAPSVFIFPPSDEQLKSGTASVVCLLNNFYPREAKVQWCVDNALQSGNSQESVTEQDSKDSTYSLSSTLTLSKADYEKHKVYACEVTHQGLSSPVTKSFNRGEC

SEQ ID NO: 69 - protein, 138 aa, Artificial Sequence
  Synthetic Construct
ERTFVMIKPDGVQRGLIGEIISRFERKGLKIVAMKMMRISREMAEKHYAEHREKPFFSALVDYITSGPVVAMVLEGKNAVEVVRKMVGATNPKEAAPGTIRGDFGLDVGKNVIFASDSPESAEREISLFFKDEELVEW

SEQ ID NO: 70 - protein, 138 aa, Artificial Sequence
  Synthetic Construct
ERTFVMIKPDGVQRGLIGEIISRFERKGFKIVAMKLMRISQELAEKHYAEHREKPFFSGLVDFITSGPVVAMVLEGKNVVEVVRKMIGATNPKEAAPGTIRGDFGMSVGKNVIFGSDSLESAEREISLFFKDEELVEW

SEQ ID NO: 71 - protein, 154 aa, Artificial Sequence
  Synthetic Construct
STNKVNKERTFLAVKPDGVARGLVGEIIARYEKKGFVLVGLKQLVPTKDLAESHYAEHKERPFFGGLVSFITSGPVVAMVFEGKGVVASARLMIGVTNPLASAPGSIRGDFGVDVGRNIIFGSDSVESANREIALWFKPEELLTEVKPNPNLYE

SEQ ID NO: 72 - protein, 151 aa, Artificial Sequence
  Synthetic Construct
ANSERTFIAIKPDGVQRGLVGEIIKRFEQKGFRLVGLKFLQASEDLLKEHYTDLKDRPFFTGLVKYMHSGPVVAMVWEGLNVVKTGRVMLGETNPADSKPGTIRGDFCIQVGRNIIFGSDSVKSAEKEISLWFQPEELVEYKSCAQNWIYE

SEQ ID NO: 73 - protein, 151 aa, Artificial Sequence
  Synthetic Construct
ANLERTFIAIKPDGVQRGLVGEIIKRFEQKGFRLVAMKFLRASEEHLKQHYIDLKDRPFFPGLVKYMNSGPVVAMVWEGLNVVKTGRVMLGETNPADSKPGTIRGDFCIQVGRNIIFGSDSVESAEKEIHLWFKPEELIDYKSCAHDWVYE

SEQ ID NO: 74 - protein, 386 aa, Artificial Sequence
  Synthetic Construct
EVQLVESGGGLVQPGGSLRLSCAASGFTFSNTDISWVRQAPGKGLEWVGRISPSDGNTYYADSVKGRFTISADTSKNTAYLQMNSLRAEDTAVYYCARRTRWASWAFDYWGQGTLVTVSSASTKGPSVFPLAPSSKSTSGGTAALGCLVKDYFPEPVTVSWNSGALTSGVHTFPAVLQSSGLYSLSSVVTVPSSSLGTQTYICNVNHKPSNTKVDKKVEPKSCDKTHTGGGGSTNKVNKERTFLAVKPDGVARGLVGEIIARYEKKGFVLVGLKQLVPTKDLAESHYAEHKERPFFGGLVSFITSGPVVAMVFEGKGVVASARLMIGVTNPLASAPGSIRGDFGVDVGRNIIFGSDSVESANREIALWFKPEELLTEVKPNPNLYE

SEQ ID NO: 75 - protein, 6 aa, Artificial Sequence
  Synthetic Construct
CDKTHT

SEQ ID NO: 76 - protein, 6 aa, Artificial Sequence
  Synthetic Construct
CDKTHL

SEQ ID NO: 77 - protein, 5 aa, Artificial Sequence
  Synthetic Construct
CDKTH

SEQ ID NO: 78 - protein, 4 aa, Artificial Sequence
  Synthetic Construct
CDKT

SEQ ID NO: 79 - protein, 6 aa, Artificial Sequence
  Synthetic Construct
  misc_feature (6)..(6): Xaa can be any amino acid other than Thr
CDKTHX

SEQ ID NO: 80 - protein, 7 aa, Artificial Sequence
  Synthetic Construct
CDKTHTC

SEQ ID NO: 81 - protein, 10 aa, Artificial Sequence
  Synthetic Construct
CDKTHTCPPC

SEQ ID NO: 82 - protein, 10 aa, Artificial Sequence
  Synthetic Construct
CDKTHTCPPS

SEQ ID NO: 83 - protein, 10 aa, Artificial Sequence
  Synthetic Construct
CDKTHTSPPC

SEQ ID NO: 84 - protein, 10 aa, Artificial Sequence
  Synthetic Construct
CDKTHTAPPC

SEQ ID NO: 85 - protein, 10 aa, Artificial Sequence
  Synthetic Construct
CDKTHTSGGC

SEQ ID NO: 86 - protein, 6 aa, Artificial Sequence
  Synthetic Construct
CYGPPC

SEQ ID NO: 87 - protein, 4 aa, Artificial Sequence
  Synthetic Construct
CPPC

SEQ ID NO: 88 - protein, 4 aa, Artificial Sequence
  Synthetic Construct
SPPS

SEQ ID NO: 89 - protein, 232 aa, Artificial Sequence
  Synthetic Construct
EVQLVESGGGLVQPGGSLRLSCAASGFTFSNTDISWVRQAPGKGLEWVGRISPSDGNTYYADSVKGRFTISADTSKNTAYLQMNSLRAEDTAVYYCARRTRWASWAMDYWGQGTLVTVSSASTKGPSVFPLAPSSKSTSGGTAALGCLVKDYFPEPVTVSWNSGALTSGVHTFPAVLQSSGLYSLSSVVTVPSSSLGTQTYICNVNHKPSNTKVDKKVEPKSCDKTHTSPPC

SEQ ID NO: 90 - protein, 224 aa, Artificial Sequence
  Synthetic Construct
EVQLVESGGGLVQPGGSLRLSCAASGFTFSNTDISWVRQAPGKGLEWVGRISPSDGNTYYADSVKGRFTISADTSKNTAYLQMNSLRAEDTAVYYCARRTRWASWAMDYWGQGTLVTVSSASTKGPSVFPLAPSSKSTSGGTAALGCLVKDYFPEPVTVSWNSGALTSGVHTFPAVLQSSGLYSLSSVVTVPSSSLGTQTYICNVNHKPSNTKVDKKVEPKSCD

SEQ ID NO: 91 - protein, 224 aa, Artificial Sequence
  Synthetic Construct
  misc_feature (105)..(105): Xaa is Met, Leu, Lys, Phe, Tyr, Arg, Asn, Gln, His, of Trp
  misc_feature (107)..(107): Xaa is Phe, Tyr, Leu, Gln, Ile, Lys, or His
EVQLVESGGGLVQPGGSLRLSCAASGFTFSNTDISWVRQAPGKGLEWVGRISPSDGNTYYADSVKGRFTISADTSKNTAYLQMNSLRAEDTAVYYCARRTRWASXAXDYWGQGTLVTVSSASTKGPSVFPLAPSSKSTSGGTAALGCLVKDYFPEPVTVSWNSGALTSGVHTFPAVLQSSGLYSLSSVVTVPSSSLGTQTYICNVNHKPSNTKVDKKVEPKSCD

SEQ ID NO: 92 - protein, 224 aa, Artificial Sequence
  Synthetic Construct
  misc_feature (105)..(105): Xaa is Met, Leu, Lys, Phe, Tyr, Arg, Asn, Gln, His, of Trp
  misc_feature (107)..(107): Xaa is Phe, Tyr, Leu, Gln, Ile, Lys, or His
EVQLVESGGGLVQPGGSLRLSCAASGFTFSNTDISWVRQAPGKGLEWVGRISPSDGNTYYADSVKGRFTISADTSKNTAYLQMNSLRAEDTAVYYCARRTRWASXAXDYWGQGTLVTVSSASTKGPSVFPLAPSSKSTSGGTAALGCLVKDYFPEPVTVSWNSGALTSGVHTFPAVLQSSGLYSLSSVVTVPSSSLGTQTYICNVNHKPSNCKVDKKVEPKSCD